European Patent Specification EP 4 453 017 B1, published September 16, 2026. Title: PROCESSES FOR SYNTHESIZING GLUCAGON-LIKE-PEPTIDE 2 (GLP-2) ANALOGUES. Applicant: ZEALAND PHARMA A/S. The sequence listing filed with the application follows.

SEQUENCE LISTING (12 sequences)

SEQ ID NO: 1 - protein, 39 aa, synthetic construct
  REGION 1..39: note = Synthetic peptide sequence
HGEGTFSSELATILDALAARDFIAWLIATKITDKKKKKK

SEQ ID NO: 2 - protein, 36 aa, synthetic construct
  REGION 1..36: note = Synthetic peptide sequence
HGEGTFSSELATILDALAARDFIAWLIATKITDKKK

SEQ ID NO: 3 - protein, 35 aa, synthetic construct
  REGION 1..35: note = Synthetic peptide sequence
HGEGTFSSELATILDALAARDFIAWLIATKITDKK

SEQ ID NO: 4 - protein, 34 aa, synthetic construct
  REGION 1..34: note = Synthetic peptide sequence
HGEGTFSSELATILDALAARDFIAWLIATKITDK

SEQ ID NO: 5 - protein, 33 aa, synthetic construct
  REGION 1..33: note = Synthetic peptide sequence
HGEGTFSSELATILDALAARDFIAWLIATKITD

SEQ ID NO: 6 - protein, 33 aa, synthetic construct; identical to SEQ ID NO: 5
  REGION 1..33: note = Synthetic peptide sequence

SEQ ID NO: 7 - protein, 39 aa, synthetic construct
  REGION 1..39: note = Synthetic peptide sequence
HGEGSFSSELSTILDALAARDFIAWLIATKITDKKKKKK

SEQ ID NO: 8 - protein, 33 aa, synthetic construct
  REGION 1..33: note = Synthetic peptide sequence
HGEGSFSSELSTILDALAARDFIAWLIATKITD

SEQ ID NO: 9 - protein, 34 aa, synthetic construct
  REGION 1..34: note = Synthetic peptide sequence
HGEGSFSSELSTILDALAARDFIAWLIATKITDK

SEQ ID NO: 10 - protein, 33 aa, Homo sapiens
HADGSFSDEMNTILDNLAARDFINWLIQTKITD

SEQ ID NO: 11 - protein, 33 aa, synthetic construct
  REGION 1..33: note = Synthetic peptide sequence
  VARIANT 5: note = X is Ser or Thr
  VARIANT 11: note = X is Ala or Ser
HGEGXFSSELXTILDALAARDFIAWLIATKITD

SEQ ID NO: 12 - protein, 34 aa, synthetic construct
  MOD_RES 5: note = X is Ser or Thr
  MOD_RES 11: note = X is Ala or Ser
  REGION 34: note = X is Lys and is repeated 1-6 times
HGEGXFSSELXTILDALAARDFIAWLIATKITDX